European Patent Specification EP 2 760 827 B1, published July 8, 2026. Title: BROAD-SPECTRUM ANTIVIRALS AGAINST 3C OR 3C-LIKE PROTEASES OF PICORNAVIRUS-LIKE SUPERCLUSTER: PICORNAVIRUSES, CALICIVIRUSES AND CORONAVIRUSES. Applicant: Kansas State University Research Foundation The Ohio State University CHANG, KYEONG-OK KIM, YUNJEONG GROUTAS, WILLIAM  C. HUA, DUY SAIF, LINDA J. The sequence listing filed with the application follows.

SEQUENCE LISTING (21 sequences)

SEQ ID NO: 1 - protein, 14 aa, Artificial Sequence
  Synthetic substrate
EPDFHLQGPEDLAK

SEQ ID NO: 2 - protein, 14 aa, Artificial Sequence
  Synthetic substrate
KTSAVLQSGFRKME

SEQ ID NO: 3 - protein, 8 aa, Artificial Sequence
  Synthetic substrate
GLRTQSFS

SEQ ID NO: 4 - protein, 8 aa, Artificial Sequence
  Synthetic substrate
APAKQLLN

SEQ ID NO: 5 - DNA, 20 bp, Artificial Sequence
  PCR primer
  misc_feature (12)..(12): n is any base or inosine
cgytggatgcgnttycatga

SEQ ID NO: 6 - DNA, 22 bp, Artificial Sequence
  PCR primer
cttagacgccatcatcattyac

SEQ ID NO: 7 - DNA, 20 bp, Artificial Sequence
  PCR probe
  misc_feature (9)..(9): n is a or inosine
  misc_feature (12)..(12): n is c, t, or inosine
agatygcgntcncctgtcca

SEQ ID NO: 8 - DNA, 20 bp, Artificial Sequence
  PCR primer
actgcagtgactggtgcttc

SEQ ID NO: 9 - DNA, 20 bp, Artificial Sequence
  PCR primer
ccgggtttatcaacagaggt

SEQ ID NO: 10 - DNA, 24 bp, Artificial Sequence
  PCR probe
cctggtgtgatccaacctcagctg

SEQ ID NO: 11 - DNA, 18 bp, Artificial Sequence
  PCR primer
tgttcyagcctgcgtggc

SEQ ID NO: 12 - DNA, 21 bp, Artificial Sequence
  PCR primer
gaaacacggacacccaaagta

SEQ ID NO: 13 - DNA, 22 bp, Artificial Sequence
  PCR probe
tcctccggcccctgaatgyggc

SEQ ID NO: 14 - DNA, 20 bp, Artificial Sequence
  PCR primer
ttccgacgtgctcgaacttt

SEQ ID NO: 15 - DNA, 21 bp, Artificial Sequence
  PCR primer
ccaacacggttgtgacagtga

SEQ ID NO: 16 - DNA, 16 bp, Artificial Sequence
  PCR probe
tcctgaggtcaatgca

SEQ ID NO: 17 - protein, 14 aa, Norwalk virus
LPDFHLQGPEDLAR

SEQ ID NO: 18 - protein, 14 aa, Norwalk virus
QDEFQLQGPTYDFD

SEQ ID NO: 19 - protein, 14 aa, Norwalk virus
PSDAVPEGKNKGKT

SEQ ID NO: 20 - protein, 14 aa, Norwalk virus
NEKINFEAPPTLWS

SEQ ID NO: 21 - protein, 14 aa, Norwalk virus
EGETALEGGDKGHY